European Patent Application EP 4 593 019 A1, published July 30, 2025. Title: CONSTRUCTION METHOD FOR HUMANIZED ANTIBODY SEQUENCE EVALUATION MODEL AND USE THEREOF. Applicant: Nanjing GenScript Biotech Co., Ltd. Application EP PCT/CN2023/127070, filed October 27, 2023. The sequence listing filed with the application follows.

SEQUENCE LISTING (48 sequences)

SEQ ID NO: 1 - protein, 255 aa, synthetic construct
MGNSCYNIVATLLLVLNFERTRSLQDPCSNCPAGTFCDNNRNQICSPCPPNSFSSAGGQRTCDICRQCKGVFRTRKECSSTSNAECDCTPGFHCLGAGCSMCEQDCKQGQELTKKGCKDCCFGTFNDQKRGICRPWTNCSLDGKSVLVNGTKERDVVCGPSPADLSPGASSVTPPAPAREPGHSPQIISFFLALTSTALLFLLFFLTLRFSVVKRGRKKLLYIFKQPFMRPVQTTQEEDGCSCRFPEEEEGGCEL

SEQ ID NO: 2 - protein, 113 aa, synthetic construct
AAVLTQTPSPVSVTVGGTVTINCQASQSVDNNNYLAWFQQKPGQPPKQLIYSASTLASGVSSRFKGSGSGTQFTLTISGVQCDDAATYYCLGEFSASSGDWNAFGGGTEVVVK

SEQ ID NO: 3 - protein, 111 aa, synthetic construct
QSVKESEGGLFKPTDTLTLACTVSGFSLSYNAITWVRQAPGNGLEWIGVINYDGTTVYASWAKSRSTITRNTNLNTVTLKMTSLTAADTATYFCARNFNIWGPGTLVTVSS

SEQ ID NO: 4 - protein, 107 aa, synthetic construct
DIQMTQSPSSLSASVGDTVTITCRASQSISTYLSWFQQKPGKAPKLLIYVASSLQSGVPSRFSGSGSGTEFTLTIAGLQLDDLATYYCQQYNSFELSFGGGTKVDIK

SEQ ID NO: 5 - protein, 113 aa, synthetic construct
QVQLQESGPGLVKPSETLSLTCTVSGGSIDTYYWSWIRQPPGKGLEWIGYLYNPSLKSRATISLDTSKNQISLKMRSMTAADTAMYFCARDPNRAAAGAFDIWGPGTMVTVSS

SEQ ID NO: 6 - protein, 7 aa, synthetic construct
GFSLSYN

SEQ ID NO: 7 - protein, 5 aa, synthetic construct
NYDGT

SEQ ID NO: 8 - skipped

SEQ ID NO: 9 - protein, 9 aa, synthetic construct
SQSVDNNNY

SEQ ID NO: 10 - skipped

SEQ ID NO: 11 - protein, 10 aa, synthetic construct
EFSASSGDWN

SEQ ID NO: 12 - protein, 7 aa, synthetic construct
GGSIDTY

SEQ ID NO: 13 - skipped

SEQ ID NO: 14 - protein, 10 aa, synthetic construct
PNRAAAGAFD

SEQ ID NO: 15 - protein, 7 aa, synthetic construct
SQSISTY

SEQ ID NO: 16 - skipped

SEQ ID NO: 17 - protein, 6 aa, synthetic construct
YNSFEL

SEQ ID NO: 18 - protein, 113 aa, synthetic construct
DIQMTQSPSSLSASVGDTVTITCRASQSVDNNNYLSWFQQKPGKAPKLLIYSASSLQSGVPSRFSGSGSGTEFTLTIAGLQLDDLATYYCQQEFSASSGDWNSFGGGTKVDIK

SEQ ID NO: 19 - protein, 109 aa, synthetic construct
QVQLQESGPGLVKPSETLSLTCTVSGFSLSYNYWSWIRQPPGKGLEWIGNYDGTLYNPSLKSRATISLDTSKNQISLKMRSMTAADTAMYFCARDFNIWGPGTMVTVSS

SEQ ID NO: 20 - protein, 113 aa, synthetic construct; identical to SEQ ID NO: 18

SEQ ID NO: 21 - protein, 109 aa, synthetic construct; identical to SEQ ID NO: 19

SEQ ID NO: 22 - protein, 7 aa, synthetic construct
SSLQPED

SEQ ID NO: 23 - protein, 7 aa, synthetic construct
NSLQPED

SEQ ID NO: 24 - protein, 7 aa, synthetic construct
TSLQPED

SEQ ID NO: 25 - protein, 7 aa, synthetic construct
SNLQPED

SEQ ID NO: 26 - protein, 7 aa, synthetic construct
NNLQPED

SEQ ID NO: 27 - protein, 7 aa, synthetic construct
TNLQPED

SEQ ID NO: 28 - protein, 7 aa, synthetic construct
SGLQPED

SEQ ID NO: 29 - protein, 7 aa, synthetic construct
NGLQPED

SEQ ID NO: 30 - protein, 7 aa, synthetic construct
TGLQPED

SEQ ID NO: 31 - protein, 7 aa, synthetic construct
SSMQPED

SEQ ID NO: 32 - protein, 6 aa, synthetic construct
VDTSKN

SEQ ID NO: 33 - protein, 6 aa, synthetic construct
IDTSKN

SEQ ID NO: 34 - protein, 6 aa, synthetic construct
LDTSKN

SEQ ID NO: 35 - protein, 6 aa, synthetic construct
VETSKN

SEQ ID NO: 36 - protein, 6 aa, synthetic construct
IETSKN

SEQ ID NO: 37 - protein, 6 aa, synthetic construct
LETSKN

SEQ ID NO: 38 - protein, 6 aa, synthetic construct
VNTSKN

SEQ ID NO: 39 - protein, 6 aa, synthetic construct
INTSKN

SEQ ID NO: 40 - protein, 6 aa, synthetic construct
LNTSKN

SEQ ID NO: 41 - protein, 6 aa, synthetic construct
VDMSKN

SEQ ID NO: 42 - protein, 113 aa, synthetic construct
AIQMTQSPSSLSASVGDTVTITCRASQSVDNNNYLSWFQQKPGKAPKLLIYSASSLQSGVPSRFSGSGSGTEFTLTIASSLQPEDATYYCQQEFSASSGDWNSFGGGTKVDIK

SEQ ID NO: 43 - protein, 109 aa, synthetic construct
QVQLQESGPGLVKPSETLSLTCTVSGFSLSYNYWSWIRQPPGKGLEWIGNYDGTLYNPSLKSRATISLVDTSKNISLKMRSMTAADTAMYFCARDFNIWGPGTMVTVSS

SEQ ID NO: 44 - protein, 113 aa, synthetic construct
DIQMTQSPSSLSASVGDTVTITCRASQSVDNNNYLSWFQQKPGKAPKLLIYSASSLQSGVPSRFSGSGSGTEFTLTIASSLQPEDATYYCQQEFSASSGDWNSFGGGTKVDIK

SEQ ID NO: 45 - protein, 109 aa, synthetic construct; identical to SEQ ID NO: 43

SEQ ID NO: 46 - protein, 19 aa, synthetic construct
MGWSCIILFLVATATGVHS

SEQ ID NO: 47 - protein, 330 aa, synthetic construct [sequence omitted]

SEQ ID NO: 48 - protein, 107 aa, synthetic construct [sequence omitted]